European Patent Specification EP 4 041 912 B1, published May 13, 2026. Title: A NOVEL CRISPR-BASED MOLECULAR SENSING PLATFORM. Applicant: THE GOVERNING COUNCIL OF THE UNIVERSITY OF TORONTO. The sequence listing filed with the application follows.

SEQUENCE LISTING (28 sequences)

SEQ ID NO: 1 - DNA, 56 bp, Artificial Sequence
  Synthetic Construct
gcgctaatacgactcactatagggcgaagttcatatgctcaacaagggcgccgagg

SEQ ID NO: 2 - DNA, 54 bp, Artificial Sequence
  Synthetic Construct
gcgctaatacgactcactatagggcccggcgacacggtcacctttattccagtg

SEQ ID NO: 3 - DNA, 108 bp, Artificial Sequence
  Synthetic Construct
gcgctaatacgactcactataggggtctaagaactttaaataatttctactgttgtagatcaacgtcgtgactgggaagttaccgttaaaagtctaagaactttaaat

SEQ ID NO: 4 - DNA, 84 bp, Artificial Sequence
  Synthetic Construct
gcgctaatacgactcactataggggtctaagaactttaaataatttctactgttgtagatatccccctttcgccagctggcgta

SEQ ID NO: 5 - DNA, 108 bp, Artificial Sequence
  Synthetic Construct
gcgctaatacgactcactataggggtctaagaactttaaataatttctactgttgtagatcaacgtcgtgaccctggcgttaccgttaaaagtctaagaactttaaat

SEQ ID NO: 6 - DNA, 359 bp, Artificial Sequence
  Synthetic Construct
tataccatgggcagcagccatcatcatcatcatcacagcagcggcatcgaagggcgcagtgggggcggagggtccatgaccatgattacggattcactggccgtcgttttacaacgtcgtgactgggaaaaccctggcgttacccaacttaatcgccttgcagcacatccccctttcgccgattcactggccgtcgttttcaacgtcgtgactgggaaaaccctggcgttacccaacttaatcgccttgcagcacatccccctttcgccagctggcgtaatagcgaagaggcccgcaccgatcgcccttcccaacagttgcgcagcctgaatggcgaatggagtggaggaggaggcagt

SEQ ID NO: 7 - DNA, 180 bp, Artificial Sequence
  Synthetic Construct
tataccatgggcagcagccatcatcatcatcatcacagcagcggcatcgaagggcgcagtgggggcggagggtccatgaccatgattacggattcactggccgtcgttttacaacgtcgtgactgggaaaaccctggcgttacccaacttaatcgccttgcagcacatccccctttcgcc

SEQ ID NO: 8 - DNA, 180 bp, Artificial Sequence
  Synthetic Construct
actggccgtcgttttacaacgtcgtgactgggaagttacccaacttaatcgccttgcagcacatccccctttcgccagctggcgtaatagcgaagaggcccgcaccgatcgcccttcccaacagttgcgcagcctgaatggcgaaagtggaggaggaggcagtgaaaacttatacttcca

SEQ ID NO: 9 - DNA, 270 bp, Artificial Sequence
  Synthetic Construct
tataccatgggcagcagccatcatcatcatcatcacagcagcggcatcgaagggcgcagtgggggcggagggtccatgaccatgattacggattcactggccgtcgttttacaacgtcgtgactgggaaaaccctggcgttacccaacttaatcgccttgcagcacatccccctttcgccagctggcgtaatagcgaagaggcccgcaccgatcgcccttcccaacagttgcgcagcctgaatggcgaaagtggaggaggaggcagtgaa

SEQ ID NO: 10 - DNA, 274 bp, Artificial Sequence
  Synthetic Construct
ccgcgaaattaatacgactcactatagggcctctagaaataattttgtttaactttaagaaggagatataccatgaccatgattacggattcactggccgtcgttttacaacgtcgtgactgggaaaaccctggcgttacccaacttaatcgccttgcagcacatccccctttcgccagctggcgtaatagcgaagaggcccgcaccgatcgcccttcccaacagttgcgcagcctgaatggcgaataaaacccctctctaaacggaggggttt

SEQ ID NO: 11 - DNA, 108 bp, Artificial Sequence
  Synthetic Construct
gcgctaatacgactcactataggggtctaagaactttaaataatttctactgttgtagatccaactcggccgatccggccgcgagttaaaagtctaagaactttaaat

SEQ ID NO: 12 - DNA, 70 bp, Artificial Sequence
  Synthetic Construct
tgaacagccctggtcggcccttaccaactcggccgatccggccgcgaaattaatacgactcactataggg

SEQ ID NO: 13 - DNA, 180 bp, Artificial Sequence; identical to SEQ ID NO: 8
  Synthetic Construct

SEQ ID NO: 14 - DNA, 248 bp, Artificial Sequence
  Synthetic Construct
gcgctaatacgactcactatagggcgaagttcatatgctcaacaagggcgccgagggcgccatggttttcgagcctgcctatatcaaggccaatcccggcgacacggtcacctttattccagtggacaaaggacataatgtcgaatccatcaaggatatgatccgtctaagaactttaaataatttctactgttgtagatcaacgtcgtgactgggaagttaccgttaaaagtctaagaactttaaat

SEQ ID NO: 15 - DNA, 132 bp, Artificial Sequence
  Synthetic Construct.
gcgaaattaatacgactcactatagggaaataattttgtttaactttaagaaggagatataccatgaccatgattacggattcactggccgtcgttcttcagcgccgtgactgggaaaaccctggcgttacc

SEQ ID NO: 16 - DNA, 273 bp, Artificial Sequence
  Synthetic Construct
tataccatgggcagcagccatcatcatcatcatcacagcagcggcatcgaagggcgcagttgggggcggagggtccatgaccatgattacggattcactggccgtcgttttacaacgtggggtgactgggaaaaccctggcgttacccaacttaatcgccttgcagcacatccccctttcgccagctggcgtaatagcgaagaggcccgcaccgatcgcccttcccaacagttgcgcagcctgaatggcgaaagtggaggaggaggcagtgaa

SEQ ID NO: 17 - DNA, 114 bp, Artificial Sequence
  Synthetic Construct
atttaaagttcttagacttttaacggtaacttcccagtcacgacgttgatctacaacagtagaaattatttaaagttcttagacggatcatatccttgatggattcgacattat

SEQ ID NO: 18 - DNA, 114 bp, Artificial Sequence
  Synthetic Construct
atttaaagttcttagacttttaacgtaaaacgacggccagtgaatccgatctacaacagtagaaattatttaaagttcttagacggatcatatccttgatggattcgacattat

SEQ ID NO: 19 - DNA, 36 bp, Artificial Sequence
  Synthetic Construct
ccatgattacgaaggctccactgcttctgcttggga

SEQ ID NO: 20 - DNA, 135 bp, Artificial Sequence
  Synthetic Construct
gtccatgaccatgattacggattcactggccgtcgttttacaacgtcgtgactgggaaaaccctggcgttacccaacttaatcgccttgcagcacatccccctttcgccagctggcgtaatagcgaagaggcccg

SEQ ID NO: 21 - DNA, 115 bp, Artificial Sequence
  Synthetic Construct
atgattacggattcactggccgtcgttttacaacgtcgtgactgggaaaaccctggcgttacccaacttaatcgccttgcagcacatccccctttcgccagctggcgtaatagcg

SEQ ID NO: 22 - DNA, 89 bp, Artificial Sequence
  Synthetic Construct
gattacggattcactggccgtcgttttacaacgtcgtgactgggaaaaccctggcgttacccaacttaatcgccttgcagcacatcccc

SEQ ID NO: 23 - DNA, 94 bp, Artificial Sequence
  Synthetic Construct
ggattcactggccgtcgttttacaacgtcgtgactgggaaaaccctggcgttacccaacttaatcgccttgcagcacatccccctttcgccagc

SEQ ID NO: 24 - DNA, 54 bp, Artificial Sequence
  Synthetic Construct
gcgctaatacgactcactataggggacgcaaccccaggaatccgccaattcaag

SEQ ID NO: 25 - DNA, 90 bp, Artificial Sequence
  Synthetic Construct
caagcagaagcagtggagccttcgatctacaacagtagaaattatttaaagttcttagacgagcagccacattaagcatattacacacac

SEQ ID NO: 26 - DNA, 54 bp, Artificial Sequence; identical to SEQ ID NO: 24
  Synthetic Construct

SEQ ID NO: 27 - DNA, 90 bp, Artificial Sequence
  Synthetic Construct
ggtaacttcccagtcacgacgttgatctacaacagtagaaattatttaaagttcttagacgagcagccacattaagcatattacacacac

SEQ ID NO: 28 - DNA, 9 bp, Escherichia coli
aaccctggc